European Patent Specification EP 3 505 629 B1, published April 30, 2025. Title: siRNAs of Human IL-6 and Recombinant Expression CAR-T Vector and Their Construction Methods and Applications. Applicant: SHANGHAI UNICAR-THERAPY BIO-MEDICINE TECHNOLOGY CO., LTD. The sequence listing filed with the application follows.

SEQUENCE LISTING (66 sequences)

SEQ ID NO: 1 - DNA, 861 bp, Artificial sequence
  the sequence is synthetized.
atgagtattcaacatttccgtgtcgcccttattcccttttttgcggcattttgccttcctgtttttgctcacccagaaacgctggtgaaagtaaaagatgctgaagatcagttgggtgcacgagtgggttacatcgaactggatctcaacagcggtaagatccttgagagttttcgccccgaagaacgttttccaatgatgagcacttttaaagttctgctatgtggcgcggtattatcccgtattgacgccgggcaagagcaactcggtcgccgcatacactattctcagaatgacttggttgagtactcaccagtcacagaaaagcatcttacggatggcatgacagtaagagaattatgcagtgctgccataaccatgagtgataacactgcggccaacttacttctgacaacgatcggaggaccgaaggagctaaccgcttttttgcacaacatgggggatcatgtaactcgccttgatcgttgggaaccggagctgaatgaagccataccaaacgacgagcgtgacaccacgatgcctgtagcaatggcaacaacgttgcgcaaactattaactggcgaactacttactctagcttcccggcaacaattaatagactggatggaggcggataaagttgcaggaccacttctgcgctcggcccttccggctggctggtttattgctgataaatctggagccggtgagcgtgggtctcgcggtatcattgcagcactggggccagatggtaagccctcccgtatcgtagttatctacacgacggggagtcaggcaactatggatgaacgaaatagacagatcgctgagataggtgcctcactgattaagcattggtaa

SEQ ID NO: 2 - DNA, 674 bp, Artificial sequence
  the sequence is synthetized.
cccgtagaaaagatcaaaggatcttcttgagatcctttttttctgcgcgtaatctgctgcttgcaaacaaaaaaaccaccgctaccagcggtggtttgtttgccggatcaagagctaccaactctttttccgaaggtaactggcttcagcagagcgcagataccaaatactgtccttctagtgtagccgtagttaggccaccacttcaagaactctgtagcaccgcctacatacctcgctctgctaatcctgttaccagtggctgctgccagtggcgataagtcgtgtcttaccgggttggactcaagacgatagttaccggataaggcgcagcggtcgggctgaacggggggttcgtgcacacagcccagcttggagcgaacgacctacaccgaactgagatacctacagcgtgagctatgagaaagcgccacgcttcccgaagggagaaaggcggacaggtatccggtaagcggcagggtcggaacaggagagcgcacgagggagcttccagggggaaacgcctggtatctttatagtcctgtcgggtttcgccacctctgacttgagcgtcgatttttgtgatgctcgtcaggggggcggagcctatggaaaaacgccagcaacgcggcctttttacggttcctggccttttgctggccttttgctcacat

SEQ ID NO: 3 - DNA, 147 bp, Artificial sequence
  the sequence is synthetized.
atcccgcccctaactccgcccagttccgcccattctccgccccatggctgactaattttttttatttatgcagaggccgaggccgcctcggcctctgagctattccagaagtagtgaggaggcttttttggaggcctagacttttgc

SEQ ID NO: 4 - DNA, 228 bp, Artificial sequence
  the sequence is synthetized.
gtagtcttatgcaatactcttgtagtcttgcaacatggtaacgatgagttagcaacatgccttacaaggagagaaaaagcaccgtgcatgccgattggtggaagtaaggtggtacgatcgtgccttattaggaaggcaacagacgggtctgacatggattggacgaaccactgaattgccgcattgcagagatattgtatttaagtgcctagctcgatacaataaacg

SEQ ID NO: 5 - DNA, 180 bp, Artificial sequence
  the sequence is synthetized.
ggtctctctggttagaccagatctgagcctgggagctctctggctaactagggaacccactgcttaagcctcaataaagcttgccttgagtgcttcaagtagtgtgtgcccgtctgttgtgtgactctggtaactagagatccctcagacccttttagtcagtgtggaaaatctctagca

SEQ ID NO: 6 - DNA, 234 bp, Artificial sequence
  the sequence is synthetized.
tgctagagattttccacactgactaaaagggtctgagggatctctagttaccagagtcacacaacagacgggcacacactacttgaagcactcaaggcaagctttattgaggcttaagcagtgggttccctagttagccagagagctcccaggctcagatctggtctaaccagagagacccagtacaagcaaaaagcagatcttattttcgttgggagtgaattagcccttcca

SEQ ID NO: 7 - DNA, 353 bp, Artificial sequence
  the sequence is synthetized.
atgggtgcgagagcgtcagtattaagcgggggagaattagatcgcgatgggaaaaaattcggttaaggccagggggaaagaaaaaatataaattaaaacatatagtatgggcaagcagggagctagaacgattcgcagttaatcctggcctgttagaaacatcagaaggctgtagacaaatactgggacagctacaaccatcccttcagacaggatcagaagaacttagatcattatataatacagtagcaaccctctattgtgtgcatcaaaggatagagataaaagacaccaaggaagctttagacaagatagaggaagagcaaaacaaaagtaagaccaccgcacagcaa

SEQ ID NO: 8 - DNA, 233 bp, Artificial sequence
  the sequence is synthetized.
aggagctttgttccttgggttcttgggagcagcaggaagcactatgggcgcagcctcaatgacgctgacggtacaggccagacaattattgtctggtatagtgcagcagcagaacaatttgctgagggctattgaggcgcaacagcatctgttgcaactcacagtctggggcatcaagcagctccaggcaagaatcctggctgtggaaagatacctaaaggatcaacagctcc

SEQ ID NO: 9 - DNA, 489 bp, Artificial sequence
  the sequence is synthetized.
tggggatttggggttgctctggaaaactcatttgcaccactgctgtgccttggaatgctagttggagtaataaatctctggaacagattggaatcacacgacctggatggagtgggacagagaaattaacaattacacaagcttaatacactccttaattgaagaatcgcaaaaccagcaagaaaagaatgaacaagaattattggaattagataaatgggcaagtttgtggaattggtttaacataacaaattggctgtggtatataaaattattcataatgatagtaggaggcttggtaggtttaagaatagtttttgctgtactttctatagtgaatagagttaggcagggatattcaccattatcgtttcagacccacctcccaaccccgaggggacccgacaggcccgaaggaatagaagaagaaggtggagagagagacagagacagatccattcgattagtgaacggatctcgacggttaac

SEQ ID NO: 10 - DNA, 119 bp, Artificial sequence
  the sequence is synthetized.
ttttaaaagaaaaggggggattggggggtacagtgcaggggaaagaatagtagacataatagcaacagacatacaaactaaagaattacaaaaacaaattacaaaaattcaaaatttta

SEQ ID NO: 11 - DNA, 696 bp, Artificial sequence
  the sequence is synthetized.
atggcccagtccaagcacggcctgaccaaggagatgaccatgaagtaccgcatggagggctgcgtggacggccacaagttcgtgatcaccggcgagggcatcggctaccccttcaagggcaagcaggccatcaacctgtgcgtggtggagggcggccccttgcccttcgccgaggacatcttgtccgccgccttcatgtacggcaaccgcgtgttcaccgagtacccccaggacatcgtcgactacttcaagaactcctgccccgccggctacacctgggaccgctccttcctgttcgaggacggcgccgtgtgcatctgcaacgccgacatcaccgtgagcgtggaggagaactgcatgtaccacgagtccaagttctacggcgtgaacttccccgccgacggccccgtgatgaagaagatgaccgacaactgggagccctcctgcgagaagatcatccccgtgcccaagcagggcatcttgaagggcgacgtgagcatgtacctgctgctgaaggacggtggccgcttgcgctgccagttcgacaccgtgtacaaggccaagtccgtgccccgcaagatgcccgactggcacttcatccagcacaagctgacccgcgaggaccgcagcgacgccaagaaccagaagtggcacctgaccgagcacgccatcgcctccggctccgccttgccctga

SEQ ID NO: 12 - DNA, 575 bp, Artificial sequence
  the sequence is synthetized.
gcccctctccctcccccccccctaacgttactggccgaagccgcttggaataaggccggtgtgcgtttgtctatatgttattttccaccatattgccgtcttttggcaatgtgagggcccggaaacctggccctgtcttcttgacgagcattcctaggggtctttcccctctcgccaaaggaatgcaaggtctgttgaatgtcgtgaaggaagcagttcctctggaagcttcttgaagacaaacaacgtctgtagcgaccctttgcaggcagcggaaccccccacctggcgacaggtgcctctgcggccaaaagccacgtgtataagatacacctgcaaaggcggcacaaccccagtgccacgttgtgagttggatagttgtggaaagagtcaaatggctcacctcaagcgtattcaacaaggggctgaaggatgcccagaaggtaccccattgtatgggatctgatctggggcctcggtgcacatgctttacatgtgtttagtcgaggttaaaaaacgtctaggccccccgaaccacggggacgtggttttcctttgaaaaacacgatgataat

SEQ ID NO: 13 - DNA, 592 bp, Artificial sequence
  the sequence is synthetized.
aatcaacctctggattacaaaatttgtgaaagattgactggtattcttaactatgttgctccttttacgctatgtggatacgctgctttaatgcctttgtatcatgctattgcttcccgtatggctttcattttctcctccttgtataaatcctggttgctgtctctttatgaggagttgtggcccgttgtcaggcaacgtggcgtggtgtgcactgtgtttgctgacgcaacccccactggttggggcattgccaccacctgtcagctcctttccgggactttcgctttccccctccctattgccacggcggaactcatcgccgcctgccttgcccgctgctggacaggggctcggctgttgggcactgacaattccgtggtgttgtcggggaaatcatcgtcctttccttggctgctcgcctgtgttgccacctggattctgcgcgggacgtccttctgctacgtcccttcggccctcaatccagcggaccttccttcccgcggcctgctgccggctctgcggcctcttccgcgtcttcgccttcgccctcagacgagtcggatctccctttgggccgcctccccgcctg

SEQ ID NO: 14 - DNA, 256 bp, Artificial sequence
  the sequence is synthetized.
ccccttcaccgagggcctatttcccatgattccttcatatttgcatatacgatacaaggctgttagagagataattggaattaatttgactgtaaacacaaagatattagtacaaaatacgtgacgtagaaagtaataatttcttgggtagtttgcagttttaaaattatgttttaaaatggactatcatatgcttaccgtaacttgaaagtatttcgatttcttggctttatatatcttgtggaaaggacgaaac

SEQ ID NO: 15 - DNA, 1178 bp, Artificial sequence
  the sequence is synthetized.
gctccggtgcccgtcagtgggcagagcgcacatcgcccacagtccccgagaagttggggggaggggtcggcaattgaaccggtgcctagagaaggtggcgcggggtaaactgggaaagtgatgtcgtgtactggctccgcctttttcccgagggtgggggagaaccgtatataagtgcagtagtcgccgtgaacgttctttttcgcaacgggtttgccgccagaacacaggtaagtgccgtgtgtggttcccgcgggcctggcctctttacgggttatggcccttgcgtgccttgaattacttccacctggctgcagtacgtgattcttgatcccgagcttcgggttggaagtgggtgggagagttcgaggccttgcgcttaaggagccccttcgcctcgtgcttgagttgaggcctggcctgggcgctggggccgccgcgtgcgaatctggtggcaccttcgcgcctgtctcgctgctttcgataagtctctagccatttaaaatttttgatgacctgctgcgacgctttttttctggcaagatagtcttgtaaatgcgggccaagatctgcacactggtatttcggtttttggggccgcgggcggcgacggggcccgtgcgtcccagcgcacatgttcggcgaggcggggcctgcgagcgcggccaccgagaatcggacgggggtagtctcaagctggccggcctgctctggtgcctggcctcgcgccgccgtgtatcgccccgccctgggcggcaaggctggcccggtcggcaccagttgcgtgagcggaaagatggccgcttcccggccctgctgcagggagctcaaaatggaggacgcggcgctcgggagagcgggcgggtgagtcacccacacaaaggaaaagggcctttccgtcctcagccgtcgcttcatgtgactccactgagtaccgggcgccgtccaggcacctcgattagttctcgagcttttggagtacgtcgtctttaggttggggggaggggttttatgcgatggagtttccccacactgagtgggtggagactgaagttaggccagcttggcacttgatgtaattctccttggaatttgccctttttgagtttggatcttggttcattctcaagcctcagacagtggttcaaagtttttttcttccatttcaggtgtcgtga

SEQ ID NO: 16 - DNA, 63 bp, Artificial sequence
  the sequence is synthetized.
atggccttaccagtgaccgccttgctcctgccgctggccttgctgctccacgccgccaggccg

SEQ ID NO: 17 - DNA, 321 bp, Artificial sequence
  the sequence is synthetized.
gacatccagatgacacagactacatcctccctgtctgcctctctgggagacagagtcaccatcagttgcagggcaagtcaggacattagtaaatatttaaattggtatcagcagaaaccagatggaactgttaaactcctgatctaccatacatcaagattacactcaggagtcccatcaaggttcagtggcagtgggtctggaacagattattctctcaccattagcaacctggagcaagaagatattgccacttacttttgccaacagggtaatacgcttccgtacacgttcggaggggggaccaagctggagatcaca

SEQ ID NO: 18 - DNA, 45 bp, Artificial sequence
  the sequence is synthetized.
ggtggcggtggctcgggcggtggtgggtcgggtggcggcggatct

SEQ ID NO: 19 - DNA, 360 bp, Artificial sequence
  the sequence is synthetized.
gaggtgaaactgcaggagtcaggacctggcctggtggcgccctcacagagcctgtccgtcacatgcactgtctcaggggtctcattacccgactatggtgtaagctggattcgccagcctccacgaaagggtctggagtggctgggagtaatatggggtagtgaaaccacatactataattcagctctcaaatccagactgaccatcatcaaggacaactccaagagccaagttttcttaaaaatgaacagtctgcaaactgatgacacagccatttactactgtgccaaacattattactacggtggtagctatgctatggactactggggccaaggaacctcagtcaccgtctcctca

SEQ ID NO: 20 - DNA, 141 bp, Artificial sequence
  the sequence is synthetized.
accacgacgccagcgccgcgaccaccaacaccggcgcccaccatcgcgtcgcagcccctgtccctgcgcccagaggcgtgccggccagcggcggggggcgcagtgcacacgagggggctggacttcgcctgtgatatctac

SEQ ID NO: 21 - DNA, 66 bp, Artificial sequence
  the sequence is synthetized.
atctgggcgcccttggccgggacttgtggggtccttctcctgtcactggttatcaccctttactgc

SEQ ID NO: 22 - DNA, 126 bp, Artificial sequence
  the sequence is synthetized.
aaacggggcagaaagaaactcctgtatatattcaaacaaccatttatgagaccagtacaaactactcaagaggaagatggctgtagctgccgatttccagaagaagaagaaggaggatgtgaactg

SEQ ID NO: 23 - DNA, 336 bp, Artificial sequence
  the sequence is synthetized.
agagtgaagttcagcaggagcgcagacgcccccgcgtacaagcagggccagaaccagctctataacgagctcaatctaggacgaagagaggagtacgatgttttggacaagagacgtggccgggaccctgagatggggggaaagccgagaaggaagaaccctcaggaaggcctgtacaatgaactgcagaaagataagatggcggaggcctacagtgagattgggatgaaaggcgagcgccggaggggcaaggggcacgatggcctttaccagggtctcagtacagccaccaaggacacctacgacgcccttcacatgcaggccctgccccctcgc

SEQ ID NO: 24 - DNA, 123 bp, Artificial sequence
  the sequence is synthetized.
aggagtaagaggagcaggctcctgcacagtgactacatgaacatgactccccgccgccccgggcccacccgcaagcattaccagccctatgccccaccacgcgacttcgcagcctatcgctcc

SEQ ID NO: 25 - DNA, 36 bp, Artificial sequence
  the sequence is synthetized.
attcaaaattttatcgatgctccggtgcccgtcagt

SEQ ID NO: 26 - DNA, 22 bp, Artificial sequence
  the sequence is synthetized.
tcacgacacctgaaatggaaga

SEQ ID NO: 27 - DNA, 42 bp, Artificial sequence
  the sequence is synthetized.
ggtgtcgtgaggatccgccaccatggccttaccagtgaccgc

SEQ ID NO: 28 - DNA, 31 bp, Artificial sequence
  the sequence is synthetized.
gtgtcatctggatgtccggcctggcggcgtg

SEQ ID NO: 29 - DNA, 41 bp, Artificial sequence
  the sequence is synthetized.
cacgccgccaggccggacatccagatgacacagactacatc

SEQ ID NO: 30 - DNA, 20 bp, Artificial sequence
  the sequence is synthetized.
tgtgatctccagcttggtcc

SEQ ID NO: 31 - DNA, 82 bp, Artificial sequence
  the sequence is synthetized.
caagctggagatcacaggtggcggtggctcgggcggtggtgggtcgggtggcggcggatctgaggtgaaactgcaggagtca

SEQ ID NO: 32 - DNA, 21 bp, Artificial sequence
  the sequence is synthetized.
tgaggagacggtgactgaggt

SEQ ID NO: 33 - DNA, 33 bp, Artificial sequence
  the sequence is synthetized.
agtcaccgtctcctcaaccacgacgccagcgcc

SEQ ID NO: 34 - DNA, 23 bp, Artificial sequence
  the sequence is synthetized.
gtagatatcacaggcgaagtcca

SEQ ID NO: 35 - DNA, 33 bp, Artificial sequence
  the sequence is synthetized.
cgcctgtgatatctacatctgggcgcccttggc

SEQ ID NO: 36 - DNA, 39 bp, Artificial sequence
  the sequence is synthetized.
tctttctgccccgtttgcagtaaagggtgataaccagtg

SEQ ID NO: 37 - DNA, 21 bp, Artificial sequence
  the sequence is synthetized.
aaacggggcagaaagaaactc

SEQ ID NO: 38 - DNA, 40 bp, Artificial sequence
  the sequence is synthetized.
tgctgaacttcactctcagttcacatcctccttcttcttc

SEQ ID NO: 39 - DNA, 22 bp, Artificial sequence
  the sequence is synthetized.
agagtgaagttcagcaggagcg

SEQ ID NO: 40 - DNA, 34 bp, Artificial sequence
  the sequence is synthetized.
ggagaggggcgtcgacttagcgagggggcagggc

SEQ ID NO: 41 - DNA, 54 bp, Artificial sequence
  the sequence is synthetized.
ccggttctccgaacgtgtcacgtctcgagacgtgacacgttcggagaatttttg

SEQ ID NO: 42 - DNA, 54 bp, Artificial sequence
  the sequence is synthetized.
aattcaaaaattctccgaacgtgtcacgtctcgagacgtgacacgttcggagaa

SEQ ID NO: 43 - DNA, 59 bp, Artificial sequence
  the sequence is synthetized.
ccgggtgaagctgagttaatttatgctcgagtaaattaactcagcttcacatttttttg

SEQ ID NO: 44 - DNA, 59 bp, Artificial sequence
  the sequence is synthetized.
aattcaaaaaaatgtgaagctgagttaatttactcgagcataaattaactcagcttcac

SEQ ID NO: 45 - DNA, 59 bp, Artificial sequence
  the sequence is synthetized.
ccgggcacagaacttatgttgttctctcgagaacaacataagttctgtgcccttttttg

SEQ ID NO: 46 - DNA, 59 bp, Artificial sequence
  the sequence is synthetized.
aattcaaaaaagggcacagaacttatgttgttctcgagagaacaacataagttctgtgc

SEQ ID NO: 47 - DNA, 59 bp, Artificial sequence
  the sequence is synthetized.
ccggctcagattgttgttgttaatgctcgagttaacaacaacaatctgaggtttttttg

SEQ ID NO: 48 - DNA, 59 bp, Artificial sequence
  the sequence is synthetized.
aattcaaaaaaacctcagattgttgttgttaactcgagcattaacaacaacaatctgag

SEQ ID NO: 49 - DNA, 59 bp, Artificial sequence
  the sequence is synthetized.
ccgggcagctttaaggagttcctgcctcgagaggaactccttaaagctgcgcttttttg

SEQ ID NO: 50 - DNA, 59 bp, Artificial sequence
  the sequence is synthetized.
aattcaaaaaagcgcagctttaaggagttcctctcgaggcaggaactccttaaagctgc

SEQ ID NO: 51 - DNA, 59 bp, Artificial sequence
  the sequence is synthetized.
ccgggtgtaggcttacctcaaataactcgagatttgaggtaagcctacacttttttttg

SEQ ID NO: 52 - DNA, 59 bp, Artificial sequence
  the sequence is synthetized.
aattcaaaaaaaagtgtaggcttacctcaaatctcgagttatttgaggtaagcctacac

SEQ ID NO: 53 - DNA, 59 bp, Artificial sequence
  the sequence is synthetized.
ccggctcaaataaatggctaacttactcgagagttagccatttatttgaggtttttttg

SEQ ID NO: 54 - DNA, 59 bp, Artificial sequence
  the sequence is synthetized.
aattcaaaaaaacctcaaataaatggctaactctcgagtaagttagccatttatttgag

SEQ ID NO: 55 - DNA, 59 bp, Artificial sequence
  the sequence is synthetized.
ccgggatgcttccaatctggattcactcgagaatccagattggaagcatccattttttg

SEQ ID NO: 56 - DNA, 59 bp, Artificial sequence
  the sequence is synthetized.
aattcaaaaaatggatgcttccaatctggattctcgagtgaatccagattggaagcatc

SEQ ID NO: 57 - DNA, 59 bp, Artificial sequence
  the sequence is synthetized.
ccggcttccaatctggattcaatgactcgagattgaatccagattggaagcattttttg

SEQ ID NO: 58 - DNA, 59 bp, Artificial sequence
  the sequence is synthetized.
aattcaaaaaatgcttccaatctggattcaatctcgagtcattgaatccagattggaag

SEQ ID NO: 59 - DNA, 21 bp, Artificial sequence
  the sequence is synthetized.
cctttccgggactttcgcttt

SEQ ID NO: 60 - DNA, 20 bp, Artificial sequence
  the sequence is synthetized.
gcagaatccaggtggcaaca

SEQ ID NO: 61 - DNA, 21 bp, Artificial sequence
  the sequence is synthetized.
catgtacgttgctatccaggc

SEQ ID NO: 62 - DNA, 21 bp, Artificial sequence
  the sequence is synthetized.
ctccttaatgtcacgcacgat

SEQ ID NO: 63 - DNA, 21 bp, Artificial sequence
  the sequence is synthetized.
gacttgtggggtccttctcct

SEQ ID NO: 64 - DNA, 21 bp, Artificial sequence
  the sequence is synthetized.
gcagctacagccatcttcctc

SEQ ID NO: 65 - DNA, 19 bp, Artificial sequence
  the sequence is synthetized.
ggattcaatgaggagactt

SEQ ID NO: 66 - DNA, 18 bp, Artificial sequence
  the sequence is synthetized.
atctgttctggaggtact